European Patent Application EP 4 147 714 A1, published March 15, 2023. Title: Human Antibodies That Bind Lymphocyte Activation Gene-3 (LAG-3), And Uses Thereof. Applicant: E. R. Squibb & Sons, L.L.C. The sequence listing filed with the application follows.

SEQUENCE LISTING (94 sequences)

SEQ ID NO: 1 - protein, 5 aa, Homo sapiens
DYYWN

SEQ ID NO: 2 - protein, 5 aa, Homo sapiens
SYGMH

SEQ ID NO: 3 - protein, 5 aa, Homo sapiens
DYGMS

SEQ ID NO: 4 - protein, 5 aa, Homo sapiens
GYYWS

SEQ ID NO: 5 - protein, 5 aa, Homo sapiens
EVSMH

SEQ ID NO: 6 - protein, 5 aa, Homo sapiens
SYGMH

SEQ ID NO: 7 - protein, 16 aa, Homo sapiens
EINHNGNTNSNPSLKS

SEQ ID NO: 8 - protein, 17 aa, Homo sapiens
VIWYDGSNKYYADSVKG

SEQ ID NO: 9 - protein, 17 aa, Homo sapiens
GINWNGGSTYYADSVKG

SEQ ID NO: 10 - protein, 16 aa, Homo sapiens
EINHRGNTNCNPSLKS

SEQ ID NO: 11 - protein, 17 aa, Homo sapiens
GFDPEDGETIYAQKFQG

SEQ ID NO: 12 - protein, 17 aa, Homo sapiens
VIWYDGSNKYYADSVKG

SEQ ID NO: 13 - protein, 12 aa, Homo sapiens
GYSDYEYNWFDP

SEQ ID NO: 14 - protein, 13 aa, Homo sapiens
EWAVASWDYGMDV

SEQ ID NO: 15 - protein, 5 aa, Homo sapiens
PVGVV

SEQ ID NO: 16 - protein, 12 aa, Homo sapiens
GYDILTGYYEDS

SEQ ID NO: 17 - protein, 11 aa, Homo sapiens
AFVVVVAASDY

SEQ ID NO: 18 - protein, 14 aa, Homo sapiens
DPHCSSTNCYLFDY

SEQ ID NO: 19 - protein, 11 aa, Homo sapiens
RASQSISSYLA

SEQ ID NO: 20 - protein, 12 aa, Homo sapiens
RASQSVSSSYLA

SEQ ID NO: 21 - protein, 11 aa, Homo sapiens
RASQGIRSALA

SEQ ID NO: 22 - protein, 11 aa, Homo sapiens
RASQSVSSYLA

SEQ ID NO: 23 - protein, 11 aa, Homo sapiens
RASQSVSSYLA

SEQ ID NO: 24 - protein, 11 aa, Homo sapiens
RASQSVSSYLA

SEQ ID NO: 25 - protein, 7 aa, Homo sapiens
DASNRAT

SEQ ID NO: 26 - protein, 7 aa, Homo sapiens
GASSRAT

SEQ ID NO: 27 - protein, 7 aa, Homo sapiens
DASSLES

SEQ ID NO: 28 - protein, 7 aa, Homo sapiens
NASNRAT

SEQ ID NO: 29 - protein, 7 aa, Homo sapiens
DASNRAT

SEQ ID NO: 30 - protein, 7 aa, Homo sapiens
DASNRAT

SEQ ID NO: 31 - protein, 9 aa, Homo sapiens
QQRSNWPLT

SEQ ID NO: 32 - protein, 9 aa, Homo sapiens
QQYGSSPFT

SEQ ID NO: 33 - protein, 9 aa, Homo sapiens
QQFNSYPYT

SEQ ID NO: 34 - protein, 9 aa, Homo sapiens
QQRSNWPLT

SEQ ID NO: 35 - protein, 9 aa, Homo sapiens
QQRSNWPWT

SEQ ID NO: 36 - protein, 9 aa, Homo sapiens
QQRSNWPIT

SEQ ID NO: 37 - protein, 120 aa, Homo sapiens
QVQLQQWGAGLLKPSETLSLTCAVYGGSFSDYYWNWIRQPPGKGLEWIGEINHNGNTNSNPSLKSRVTLSLDTSKNQFSLKLRSVTAADTAVYYCAFGYSDYEYNWFDPWGQGTLVTVSS

SEQ ID NO: 38 - protein, 122 aa, Homo sapiens
QVQLVESGGGVVQPGRSLRLSCAASGFTFSSYGMHWVRQAPGKGLEWVAVIWYDGSNKYYADSVKGRFTISRDNSKNTLYLQMNSLRAEDTAVYYCAREWAVASWDYGMDVWGQGTTVTVSS

SEQ ID NO: 39 - protein, 112 aa, Homo sapiens
EVQLVESGGGVVRPGGSLRLSCAASGFTFDDYGMSWVRQAPGKGLEWVSGINWNGGSTYYADSVKGRFTISGDNAKNSLYLQMNSLRAEDTALYYCTTGGYWGQGTLVTVSS

SEQ ID NO: 40 - protein, 120 aa, Homo sapiens
QVQLQQWGAGLLKPSETLSLTCAVYGGSFSGYYWSWIRQPPGKGLEWIGEINHRGNTNCNPSLKSRVTISGDTSKKQFALKLNSVTAADTAVYYCARGYDILTGYYEDSWGPGTLVTVSS

SEQ ID NO: 41 - protein, 123 aa, Homo sapiens
THDQVQLVQSGAEVKKPGASVKVSCKVSGYTLTEVSMHWVRQAPGKGLEWMGGFDPEDGETIYAQKFQGRVTMTEDTSTDTAYMELSSLRSEDTAVYYCATAFVVVVAASDYWGQGTLVTVSS

SEQ ID NO: 42 - protein, 123 aa, Homo sapiens
QVHLVESGGGVVQPGRSLRLSCAASGFTFSSYGMHWVRQAPGKGLEWVAVIWYDGSNKYYADSVKGRFTISRDNSKNTLYLQMNSLRAEDTAVYYCARDPHCSSTNCYLFDYWGQGTLVTVSS

SEQ ID NO: 43 - protein, 107 aa, Homo sapiens
EIVLTQSPATLSLSPGERATLSCRASQSISSYLAWYQQKPGQAPRLLIYDASNRATGIPARFSGSGSGTDFTLTISSLEPEDFAVYYCQQRSNWPLTFGQGTNLEIK

SEQ ID NO: 44 - protein, 108 aa, Homo sapiens
EIVLTQSPGTLSLSPGERATLSCRASQSVSSSYLAWYQQKPGQAPRLLIYGASSRATGIPDRFSGSGSGTDFTLTISRLEPEDFAVYYCQQYGSSPFTFGPGTKVDIK

SEQ ID NO: 45 - protein, 107 aa, Homo sapiens
AIQLTQSPSSLSASVGDRVTITCRASQGIRSALAWYQQKPGKAPKLLIYDASSLESGVPSRFSGSGSGTDFTLTISSLQPEDFATYYCQQFNSYPYTFGQGTKLEIK

SEQ ID NO: 46 - protein, 107 aa, Homo sapiens
EIVLTQSPATLSLSPGERATLSCRASQSVSSYLAWYQQKPGQAPRLLIYNASNRATGIPARFSGSGSGTDFTLTISSLEPEDFAVYYCQQRSNWPLTFGGGTKVEIK

SEQ ID NO: 47 - protein, 107 aa, Homo sapiens
EIVLTQSPATLSLSPGERATLSCRASQSVSSYLAWYQQKPGQAPRLLIYDASNRATGIPARFSGSGSGTDFTLTISSLEPEDFAVYYCQQRSNWPWTFGQGTKVEIK

SEQ ID NO: 48 - protein, 107 aa, Homo sapiens
EIVLTQSPATLSLSPGERATLSCRASQSVSSYLAWYQQKPGQAPRLLIYDASNRATGIPARFSGSGSGTDFTLTISSLEPEDFAVYYCQQRSNWPITFGQGTRLEIK

SEQ ID NO: 49 - DNA, 360 bp, Homo sapiens
  source 1..360: mol_type = other DNA
caggtgcagctacagcagtggggcgcaggactgttgaagccttcggagaccctgtccctcacctgcgctgtctatggtgggtccttcagtgattactactggaactggatccgccagcccccagggaaggggctggagtggattggggaaatcaatcataatggaaacaccaactccaacccgtccctcaagagtcgagtcaccctatcactagacacgtccaagaaccagttctccctgaagctgaggtctgtgaccgccgcggacacggctgtgtattactgtgcgtttggatatagtgactacgagtacaactggttcgacccctggggccagggaaccctggtcaccgtctcctca

SEQ ID NO: 50 - DNA, 366 bp, Homo sapiens
  source 1..366: mol_type = other DNA
caggtgcagctggtggagtctgggggaggcgtggtccagcctgggaggtccctgagactctcctgtgcagcgtctggattcaccttcagtagctatggcatgcactgggtccgccaggctccaggcaaggggctggagtgggtggcagttatatggtatgatggaagtaataaatactatgcagactccgtgaagggccgattcaccatctccagagacaattccaagaacacgctgtatctgcaaatgaacagcctgagagccgaggacacggctgtgtattactgtgcgagagaatgggcagtggcctcctgggactacggtatggacgtctggggccaagggaccacggtcaccgtctcctca

SEQ ID NO: 51 - DNA, 336 bp, Homo sapiens
  source 1..336: mol_type = other DNA
gaggtgcagttggtggagtctgggggaggtgtggtacggcctggggggtccctgagactctcctgtgcagcctctggattcacctttgatgattatggcatgagctgggtccgccaagctccagggaaggggctggagtgggtctctggtattaattggaatggtggtagcacatattatgcagactctgtgaagggccgattcaccatctccggagacaacgccaagaactccctgtatctgcaaatgaacagtctgagagccgaggacacggccttgtattactgtaccactgggggctactggggccagggaaccctggtcaccgtctcctca

SEQ ID NO: 52 - DNA, 360 bp, Homo sapiens
  source 1..360: mol_type = other DNA
caggtgcagctacagcagtggggcgcaggactgttgaagccatcggaaaccctgtccctcacctgcgctgtctatggtgggtccttcagtggttactactggagctggatccgccagcccccagggaaggggctggagtggattggggaaatcaatcatcgtggaaacaccaactgcaacccgtccctcaagagtcgagtcaccatatcaggagatacgtccaagaaacagttcgccctgaagctgaactctgtgaccgccgcggacacggctgtctattactgtgcgagaggatacgatattttgactggttattatgaggactcctggggcccgggaaccctggtcaccgtctcctca

SEQ ID NO: 53 - DNA, 369 bp, Homo sapiens
  source 1..369: mol_type = other DNA
acccacgaccaggtccagctggtacagtctggggctgaggtgaagaagcctggggcctcagtgaaggtctcctgcaaggtttccggatacaccctcactgaagtatccatgcactgggtgcgacaggctcctggaaaagggcttgagtggatgggaggttttgatcctgaagatggtgaaacaatctacgcacagaagttccagggcagagtcaccatgaccgaggacacatctacagacacagcctacatggagctgagcagcctgagatctgaggacacggccgtgtattactgtgcaacagcctttgtagtggtggtagctgcttctgactactggggccagggaaccctggtcaccgtctcctca

SEQ ID NO: 54 - DNA, 369 bp, Homo sapiens
  source 1..369: mol_type = other DNA
caggtgcacctggtggagtctgggggaggcgtggtccagcctgggaggtccctgagactctcctgtgcagcgtctggattcaccttcagtagctatggcatgcactgggtccgccaggctccaggcaaggggctggagtgggtggcagttatatggtatgatggaagtaataaatactatgcagactccgtgaagggccgattcaccatctccagagacaattccaagaacacgctgtatctgcaaatgaacagcctgagagccgaggacacggctgtgtattactgtgcgagagatccccattgtagtagtaccaactgctacctttttgactactggggccagggaaccctggtcaccgtctcctca

SEQ ID NO: 55 - DNA, 321 bp, Homo sapiens
  source 1..321: mol_type = other DNA
gaaattgtgttgacacagtctccagccaccctgtctttgtctccaggggaaagagccaccctctcctgcagggccagtcagagtattagcagctacttagcctggtaccaacagaaacctggccaggctcccaggctcctcatctatgatgcatccaacagggccactggcatcccagccaggttcagtggcagtgggtctgggacagacttcactctcaccatcagcagcctagagcctgaagattttgcagtttattactgtcagcagcgtagcaactggcctctcacttttggccaggggaccaacctggagatcaaa

SEQ ID NO: 56 - DNA, 324 bp, Homo sapiens
  source 1..324: mol_type = other DNA
gaaattgtgttgacgcagtctccaggcaccctgtctttgtctccaggggaaagagccaccctctcctgcagggccagtcagagtgttagcagcagctacttagcctggtaccagcagaaacctggccaggctcccaggctcctcatctatggtgcatccagcagggccactggcatcccagacaggttcagtggcagtgggtctgggacagacttcactctcaccatcagcagactggagcctgaagattttgcagtgtattactgtcagcagtatggtagctcaccattcactttcggccctgggaccaaagtggatatcaaa

SEQ ID NO: 57 - DNA, 321 bp, Homo sapiens
  source 1..321: mol_type = other DNA
gccatccagttgacccagtctccatcctccctgtctgcatctgtaggagacagagtcaccatcacttgccgggcaagtcagggcattaggagtgctttagcctggtatcagcagaaaccagggaaagctcctaagctcctgatctatgatgcctccagtttggaaagtggggtcccatcaaggttcagcggcagtggatctgggacagatttcactctcaccatcagcagcctgcagcctgaagattttgcaacttattactgtcaacagtttaatagttacccgtacacttttggccaggggaccaagctggagatcaaa

SEQ ID NO: 58 - DNA, 321 bp, Homo sapiens
  source 1..321: mol_type = other DNA
gaaattgtgttgacacagtctccagccaccctgtctttgtctccaggggaaagagccaccctctcctgcagggccagtcagagtgttagcagctacttagcctggtaccaacagaaacctggccaggctcccaggctcctcatctataatgcatccaacagggccactggcatcccagccaggttcagtggcagtgggtctgggacagacttcactctcaccatcagcagcctagagcctgaagattttgcagtttattactgtcagcagcgtagcaactggccgctcactttcggcggagggaccaaggtggagatcaaa

SEQ ID NO: 59 - DNA, 321 bp, Homo sapiens
  source 1..321: mol_type = other DNA
gaaattgtgttgacacagtctccagccaccctgtctttgtctccaggggaaagagccaccctctcctgcagggccagtcagagtgttagcagctacttagcctggtaccaacagaaacctggccaggctcccaggctcctcatctatgatgcatccaacagggccactggcatcccagccaggttcagtggcagtgggtctgggacagacttcactctcaccatcagcagcctagagcctgaagattttgcagtttattactgtcagcagcgtagcaactggccgtggacgttcggccaagggaccaaggtggaaatcaaa

SEQ ID NO: 60 - DNA, 321 bp, Homo sapiens
  source 1..321: mol_type = other DNA
gaaattgtgttgacacagtctccagccaccctgtctttgtctccaggggaaagagccaccctctcctgcagggccagtcagagtgttagcagctacttagcctggtaccaacagaaacctggccaggctcccaggctcctcatctatgatgcatccaacagggccactggcatcccagccaggttcagtggcagtgggtctgggacagacttcactctcaccatcagcagcctagagcctgaagattttgcagtttattactgtcagcagcgtagcaactggcctatcaccttcggccaagggacacgactggagattaaa

SEQ ID NO: 61 - protein, 98 aa, Homo sapiens
  SITE 98: note = MISC_FEATURE - Residue 98 is presented only in a subset of figures.
QVQLQQWGAGLLKPSETLSLTCAVYGGSFSGYYWSWIRQPPGKGLEWIGEINHSGSTNYNPSLKSRVTISVDTSKNQFSLKLSSVTAADTAVYYCARG

SEQ ID NO: 62 - protein, 16 aa, Homo sapiens
  REGION 1..3: note = MISC_FEATURE - Residues 1-3 are presented only in a subset of figures.
NWFDPWGQGTLVTVSS

SEQ ID NO: 63 - protein, 95 aa, Homo sapiens
EIVLTQSPATLSLSPGERATLSCRASQSVSSYLAWYQQKPGQAPRLLIYDASNRATGIPARFSGSGSGTDFTLTISSLEPEDFAVYYCQQRSNWP

SEQ ID NO: 64 - protein, 12 aa, Homo sapiens
  SITE 1: note = MISC_FEATURE - Residue 1 is presented only in a subset of figures.
YTFGQGTKLEIK

SEQ ID NO: 65 - protein, 98 aa, Homo sapiens
QVQLVESGGGVVQPGRSLRLSCAASGFTFSSYGMHWVRQAPGKGLEWVAVIWYDGSNKYYADSVKGRFTISRDNSKNTLYLQMNSLRAEDTAVYYCAR

SEQ ID NO: 66 - protein, 16 aa, Homo sapiens
YGMDVWGQGTTVTVSS

SEQ ID NO: 67 - protein, 96 aa, Homo sapiens
EIVLTQSPGTLSLSPGERATLSCRASQSVSSSYLAWYQQKPGQAPRLLIYGASSRATGIPDRFSGSGSGTDFTLTISRLEPEDFAVYYCQQYGSSP

SEQ ID NO: 68 - protein, 12 aa, Homo sapiens
FTFGPGTKVDIK

SEQ ID NO: 69 - protein, 98 aa, Homo sapiens
EVQLVESGGGVVRPGGSLRLSCAASGFTFDDYGMSWVRQAPGKGLEWVSGINWNGGSTGYADSVKGRFTISRDNAKNSLYLQMNSLRAEDTALYHCAR

SEQ ID NO: 70 - protein, 14 aa, Homo sapiens
  REGION 1..2: note = MISC_FEATURE - Residues 1-2 are only presented in a subset of figures.
FDYWGQGTLVTVSS

SEQ ID NO: 71 - protein, 95 aa, Homo sapiens
AIQLTQSPSSLSASVGDRVTITCRASQGISSALAWYQQKPGKAPKLLIYDASSLESGVPSRFSGSGSGTDFTLTISSLQPEDFATYYCQQFNSYP

SEQ ID NO: 72 - protein, 12 aa, Homo sapiens
LTFGGGTKVEIK

SEQ ID NO: 73 - protein, 101 aa, Homo sapiens
THAQVQLVQSGAEVKKPGASVKVSCKVSGYTLTELSMHWVRQAPGKGLEWMGGFDPEDGETIYAQKFQGRVTMTEDTSTDTAYMELSSLRSEDTAVYYCAT

SEQ ID NO: 74 - protein, 12 aa, Homo sapiens
WTFGQGTKVEIK

SEQ ID NO: 75 - protein, 12 aa, Homo sapiens
ITFGQGTRLEIK

SEQ ID NO: 76 - protein, 8 aa, Homo sapiens
PGHPLAPG

SEQ ID NO: 77 - protein, 8 aa, Homo sapiens
HPAAPSSW

SEQ ID NO: 78 - protein, 8 aa, Homo sapiens
PAAPSSWG

SEQ ID NO: 79 - protein, 30 aa, Homo sapiens
GPPAAAPGHPLAPGPHPAAPSSWGPRPRRY

SEQ ID NO: 80 - protein, 12 aa, Homo sapiens
GPPAAAPGHPLA

SEQ ID NO: 81 - protein, 12 aa, Homo sapiens
PAAAPGHPLAPG

SEQ ID NO: 82 - protein, 12 aa, Homo sapiens
AAPGHPLAPGPH

SEQ ID NO: 83 - protein, 12 aa, Homo sapiens
PGHPLAPGPHPA

SEQ ID NO: 84 - protein, 12 aa, Homo sapiens
HPLAPGPHPAAP

SEQ ID NO: 85 - protein, 12 aa, Homo sapiens
LAPGPHPAAPSS

SEQ ID NO: 86 - protein, 12 aa, Homo sapiens
PGPHPAAPSSWG

SEQ ID NO: 87 - protein, 12 aa, Homo sapiens
PHPAAPSSWGPR

SEQ ID NO: 88 - protein, 12 aa, Homo sapiens
PAAPSSWGPRPR

SEQ ID NO: 89 - protein, 12 aa, Homo sapiens
APSSWGPRPRRY

SEQ ID NO: 90 - protein, 30 aa, Macaca sp.
GPPAPAPGHPPAPGHRPAAPYSWGPRPRRY

SEQ ID NO: 91 - DNA, 21 bp, synthetic construct
  misc_feature 1..21: note = 5Mcyn1408 primer
  source 1..21: mol_type = other DNA
atgtgggaggctcagttcctg

SEQ ID NO: 92 - DNA, 19 bp, synthetic construct
  misc_feature 1..19: note = 3Mcyn1408a primer
  source 1..19: mol_type = other DNA
gtcagagctgctccggctc

SEQ ID NO: 93 - protein, 532 aa, Macaca mulatta
MWEAQFLGLLFLQPLWVAPVKPPQPGAEISVVWAQEGAPAQLPCSPTIPLQDLSLLRRAGVTWQHQPDSGPPAPAPGHPPAPGHRPAAPYSWGPRPRRYTVLSVGPGGLRSGRLPLQPRVQLDERGRQRGDFSLWLRPARRADAGEYRATVHLRDRALSCRLRLRVGQASMTASPPGSLRTSDWVILNCSFSRPDRPASVHWFRSRGQGRVPVQGSPHHHLAESFLFLPHVGPMDSGLWGCILTYRDGFNVSIMYNLTVLGLEPATPLVYAGAGSRVELPCRLPPAVGTQSFLTAKWAPPGGGPDLLVAGDNGDFTLRLEDVSQAQAGTYICHIRLQGQQLNATVTLAIITVTPKSFGSPGSLGKLLCEVTPASGQEHFVWSPLNTPSQRSFSGPWLEAQEAQLLSQPWQCQLHQGERLLGAAVYFTELSSPGAQRSGRAPGALRAGHLPLFLILGVLFLLLLVTGAFGFHLWRRQWRPRRFSALEQGIHPPQAQSKIEELEQEPELEPEPELERELGPEPEPGPEPEPEQL

SEQ ID NO: 94 - protein, 533 aa, Macaca mulatta
MWEAQFLGLLFLQPLWVAPVKPPQPGAEISVVWAQEGAPAQLPCSPTIPLQDLSLLRRAGVTWQHQPDSGPPAPAPGHPPAPGHRPAAPYSWGPRPRRYTVLSVGPGGLRSGRLPLQPRVQLDERGRQRGDFSLWLRPARRADAGEYRATVHLRDRALSCRLRLRVGQASMTASPPGSLRTSDWVILNCSFSRPDRPASVHWFRSRGQGRVPVQGSPHHHLAESFLFLPHVGPMDSGLWGCILTYRDGFNVSIMYNLTVLGLEPATPLTVYAGAGSRVELPCRLPPAVGTQSFLTAKWAPPGGGPDLLVAGDNGDFTLRLEDVSQAQAGTYICHIRLQGQQLNATVTLAIITVTPKSFGSPGSLGKLLCEVTPASGQEHFVWSPLNTPSQRSFSGPWLEAQEAQLLSQPWQCQLHQGETLLGAAVYFTELSSPGAQRSGRAPGALRAGHLPLFLILGVLFLLLLVTGAFGFHLWRRQWRPRRFSALEQGIHPPQAQSKIEELEQEPELEPEPELERELGPEPEPGPEPEPEQL